European Patent Specification EP 3 288 547 B1, published June 7, 2023. Title: EGR1 TARGETING MOLECULES FOR THE TREATMENT OF INFLAMMATORY AND HYPERPROLIFERATIVE CONDITIONS. Applicant: The Medical Research, Infrastructure and Health Services Fund of the Tel Aviv Medical Center SARIG, Ofer SPRECHER, Eli. The sequence listing filed with the application follows.

SEQUENCE LISTING (5 sequences)

SEQ ID NO: 1 - DNA, 22 bp, Artificial Sequence
  Single strand DNA oligonucleotide
cgagcaaggtccttccatagtg

SEQ ID NO: 2 - DNA, 21 bp, Artificial Sequence
  Single strand DNA oligonucleotide
ccgatgacctcacagctcaag

SEQ ID NO: 3 - DNA, 19 bp, Artificial Sequence
  Single strand DNA oligonucleotide
gggcagtcgagtggtttgg

SEQ ID NO: 4 - DNA, 22 bp, Artificial Sequence
  Single strand DNA oligonucleotide
ttgccgacaggatgcagaagga

SEQ ID NO: 5 - DNA, 585 bp, Artificial Sequence
  A DNA fragment spanning 585bp upstream to the SAMD9 predicted transcription start site (TSS)
cctgacactgaccttagaaaagataaatctctacaatgtgaccatcaggtctgctgcagccctggtctgctctgcaataaatgaatttagcacttattggggtgctcaaagaagtcctatccctgaaagacattctttacactttaggaaaacaggaatggacagtaactccacccttaaaggccagtgaaatattgacctagagtatctccaacctggtgctctacaaggctgggactgcaatgtaaactcatattcccaagggatcaattaagccagaatatcccacagtttgtctataacaagacaatggggctttctgcagccctcaaaactctcaagtgaggaaaaattgttaagccttcagattttaaccaagcagaccagaaggtggtatatagccatagcttattaaaaagcatttcagatagaaaaggcggtgctgtaatttcagatctgagaaatgaaactgaaaccaaacctatattcttccttccccaacctcccagttgttaaacacgccctgctgtttctgagccaattagagcttgctgtgagacagaagcagagaatacatagacttcc